European Patent Application EP 4 177 266 A1, published May 10, 2023. Title: NEUTRALIZING ANTI-SARS-COV-2 HUMAN ANTIBODIES. Applicant: Katholieke Universiteit Leuven. The sequence listing filed with the application follows.

SEQUENCE LISTING (72 sequences)

SEQ ID NO: 1 - protein, 8 aa, Homo sapiens
GYTFTSHY

SEQ ID NO: 2 - protein, 8 aa, Homo sapiens
IDSSGGGA

SEQ ID NO: 3 - protein, 14 aa, Homo sapiens
AKAHSTNWYGWFDP

SEQ ID NO: 4 - protein, 8 aa, Homo sapiens
SSNIGSNT

SEQ ID NO: 5 - protein, 13 aa, Homo sapiens
AAWDDGLNGSGWV

SEQ ID NO: 6 - protein, 8 aa, Homo sapiens
GVIVSRNY

SEQ ID NO: 7 - protein, 7 aa, Homo sapiens
IYSGGST

SEQ ID NO: 8 - protein, 22 aa, Homo sapiens
ARWGPNYYGSGSDHYNSYGMDV

SEQ ID NO: 9 - protein, 7 aa, Homo sapiens
QGVSSSS

SEQ ID NO: 10 - protein, 10 aa, Homo sapiens
QQSGSSPQYT

SEQ ID NO: 11 - protein, 8 aa, Homo sapiens
GFTFDDYA

SEQ ID NO: 12 - protein, 8 aa, Homo sapiens
VSWNSGTI

SEQ ID NO: 13 - protein, 18 aa, Homo sapiens
AKDVSVYRFREQSYGMDV

SEQ ID NO: 14 - protein, 9 aa, Homo sapiens
SSDIGGYNF

SEQ ID NO: 15 - protein, 10 aa, Homo sapiens
SSYTSSSLVV

SEQ ID NO: 16 - protein, 8 aa, Homo sapiens
GFSLDDYG

SEQ ID NO: 17 - protein, 8 aa, Homo sapiens
ISWNSGDR

SEQ ID NO: 18 - protein, 18 aa, Homo sapiens
AKGSGAHYDIMTGARLDY

SEQ ID NO: 19 - protein, 6 aa, Homo sapiens
QSITNY

SEQ ID NO: 20 - protein, 9 aa, Homo sapiens
QQSYSTPWT

SEQ ID NO: 21 - DNA, 363 bp, Homo sapiens
  CDS (1)..(363)
caggtgcagctggtgcagtctggggctgaggtgaagaagcctggggcctcagtgaaggtttcctgcaaggcatatggatacaccttcaccagccactatatgcactgggtgcgacaggcccctggacaagggcttgagtggatgggaataatcgactctagtggtggtggcgcaagctacccacagaagttccagggcagagtcaccctgaccagggacacgtcctcgagcacagtctacatggagctgagcagcctgagatctgaggacacggccgtctattactgtgcgaaagcgcatagcaccaactggtacggctggttcgacccctggggccagggaaccctggtcaccgtctcctca

SEQ ID NO: 22 - protein, 121 aa, Homo sapiens
QVQLVQSGAEVKKPGASVKVSCKAYGYTFTSHYMHWVRQAPGQGLEWMGIIDSSGGGASYPQKFQGRVTLTRDTSSSTVYMELSSLRSEDTAVYYCAKAHSTNWYGWFDPWGQGTLVTVSS

SEQ ID NO: 23 - DNA, 337 bp, Homo sapiens
  CDS (1)..(336)
cagtctgtgctgactcagccaccctcaacgtctgggacccccgggcagagggtcaccatctcttgttctggaagcagctccaacatcggaagtaatactgtaaactggtaccagcagctcccaggaacggcccccaaactcctcatctataataataatcagcggccctcgggggtccctgaccgattctctggctccaagtctggcacctcagcctccctggccatcagtgggctccagtctgaggatgaggctgattattactgtgcagcatgggatgacggcctgaatggctccgggtgggtgttcggcggagggaccaagctgaccgtcctag

SEQ ID NO: 24 - protein, 112 aa, Homo sapiens
QSVLTQPPSTSGTPGQRVTISCSGSSSNIGSNTVNWYQQLPGTAPKLLIYNNNQRPSGVPDRFSGSKSGTSASLAISGLQSEDEADYYCAAWDDGLNGSGWVFGGGTKLTVL

SEQ ID NO: 25 - DNA, 384 bp, Homo sapiens
  CDS (1)..(384)
gaggtgcggctggtggagtctggaggaggcttgatccagccgggggggtccctgacactctcctgtgcagcctctggggtcatcgtcagtcgcaactacatgaactgggtccgccaggctccagggaaggggctggagtgggtctcagttatttacagcggtggtagtacattctacgcagactccgtgaagggccgattcaccatctccagagacaattccaagaacacgttgtatcttcaaatgaacagcctgagagccgaggacacggccgtgtattactgtgcgagatggggcccgaattactatggttcggggagtgatcactacaactcctacggtatggacgtctggggccaagggaccacggtcaccgtctcctca

SEQ ID NO: 26 - protein, 128 aa, Homo sapiens
EVRLVESGGGLIQPGGSLTLSCAASGVIVSRNYMNWVRQAPGKGLEWVSVIYSGGSTFYADSVKGRFTISRDNSKNTLYLQMNSLRAEDTAVYYCARWGPNYYGSGSDHYNSYGMDVWGQGTTVTVSS

SEQ ID NO: 27 - DNA, 328 bp, Homo sapiens
  CDS (1)..(327)
gaaattgtgttgacgcagtctccaggcaccctgtctttgtctccaggggaaagcgccaccctctcctgcagggccagtcagggtgttagcagcagctccttagcctggtaccagcagagacctggccaggctcccaggctcctcatgtatggtgcatccagcagggccactggcatcccagacaggttcagtggcagtgggtctgggacagacttcactctcaccatcagcagactagagcctgaagattttgcagtgtattactgtcagcagtctggtagctcacctcagtacacttttggccaggggaccaagctggagatcaaac

SEQ ID NO: 28 - protein, 109 aa, Homo sapiens
EIVLTQSPGTLSLSPGESATLSCRASQGVSSSSLAWYQQRPGQAPRLLMYGASSRATGIPDRFSGSGSGTDFTLTISRLEPEDFAVYYCQQSGSSPQYTFGQGTKLEIK

SEQ ID NO: 29 - DNA, 375 bp, Homo sapiens
  CDS (1)..(375)
gaagtgcagctggtggagtctgggggaggcttggtacagcctggcaggtccctgagactctcctgtgcagcctctggattcacctttgatgattatgccatgcactgggtccggcaagctccagggaagggcctggagtgggtctcaggtgttagttggaatagtggtaccataggctatgcggactctgtgaagggccgattcatcatctccagagacaacgccaagaactccctgtatctgcaaatgcgcagtctgagagctgaggacacggccttgtattactgtgcaaaagatgtatctgtctaccgttttagggagcagtcctacggtatggacgtctggggccaggggaccacggtcaccgtcttgtca

SEQ ID NO: 30 - protein, 125 aa, Homo sapiens
EVQLVESGGGLVQPGRSLRLSCAASGFTFDDYAMHWVRQAPGKGLEWVSGVSWNSGTIGYADSVKGRFIISRDNAKNSLYLQMRSLRAEDTALYYCAKDVSVYRFREQSYGMDVWGQGTTVTVLS

SEQ ID NO: 31 - DNA, 331 bp, Homo sapiens
  CDS (1)..(330)
cagtctgccctgactcagtctgcctccgtgtctgggtctcctggacagtcgatcaccatctcctgcactggaaccagcagtgacattggtggttataactttgtctcgtggtaccaacagcaccctggcaaagcccccaaactcatgatttatgaggtcactactcggccctcaggggtttctaatcgcttctctggctccaagtctggcaacacggcctccctgaccatctctgggctccaggctgaggacgaggctgattattactgcagctcatatacaagcagcagccttgtggtattcggcggagggaccaagctggccctcctgg

SEQ ID NO: 32 - protein, 110 aa, Homo sapiens
QSALTQSASVSGSPGQSITISCTGTSSDIGGYNFVSWYQQHPGKAPKLMIYEVTTRPSGVSNRFSGSKSGNTASLTISGLQAEDEADYYCSSYTSSSLVVFGGGTKLALL

SEQ ID NO: 33 - DNA, 375 bp, Homo sapiens
  CDS (1)..(375)
gaagtgcagctggtggagtctgggggaggcttggtacagcctggcaggtccctgagactctcctgtgcagcctctggattcagcctcgatgattatggcatgcactgggtccggcaagctccagggaagggcctggagtgggtctcaggtattagttggaatagtggtgacagaggctatgcggactctgtgaagggccgatttaccatctccagagacaacgccaagaactccctgtatctgcaaatgaacagtctgagagctgaggacacggccttgtattactgtgcaaaagggtccggcgctcactacgatatcatgactggtgctcgccttgactactggggccagggaaccctggtcaccgtctcctca

SEQ ID NO: 34 - protein, 125 aa, Homo sapiens
EVQLVESGGGLVQPGRSLRLSCAASGFSLDDYGMHWVRQAPGKGLEWVSGISWNSGDRGYADSVKGRFTISRDNAKNSLYLQMNSLRAEDTALYYCAKGSGAHYDIMTGARLDYWGQGTLVTVSS

SEQ ID NO: 35 - DNA, 322 bp, Homo sapiens
  CDS (1)..(321)
gacatccagatgacccagtctccatcctccctgtctgcatctgtaggagacagagtcaccatcacttgccgggcaagtcagagcattaccaactatttaaattggtatcagcagaaaccagggaaagtccctaagctcctgatctatgctgcatccattttgcaaagtggggtcccatcaaggttcagtggcagtggatctgggacagatttcactctcaccatcagcagtctgcaacctgaagattttgcaacttactactgtcaacagagttacagtaccccctggacgttcggccaagggaccaaggtggaaatcaaac

SEQ ID NO: 36 - protein, 107 aa, Homo sapiens
DIQMTQSPSSLSASVGDRVTITCRASQSITNYLNWYQQKPGKVPKLLIYAASILQSGVPSRFSGSGSGTDFTLTISSLQPEDFATYYCQQSYSTPWTFGQGTKVEIK

SEQ ID NO: 37 - protein, 8 aa, homo sapiens
GYSFTSHW

SEQ ID NO: 38 - protein, 8 aa, homo sapiens
IFPGDSKT

SEQ ID NO: 39 - protein, 21 aa, homo sapiens
ARPNRYYDDSGNYDGSYYFDY

SEQ ID NO: 40 - protein, 6 aa, homo sapiens
QSVNTN

SEQ ID NO: 41 - protein, 11 aa, homo sapiens
QQYNNWPPAWT

SEQ ID NO: 42 - protein, 8 aa, homo sapiens
GYTFTTYY

SEQ ID NO: 43 - protein, 8 aa, homo sapiens
INSSGGST

SEQ ID NO: 44 - protein, 12 aa, homo sapiens
ATSGWYRGAFDY

SEQ ID NO: 45 - protein, 8 aa, homo sapiens
SGSIDNNY

SEQ ID NO: 46 - protein, 9 aa, homo sapiens
QSIDSNSWV

SEQ ID NO: 47 - protein, 8 aa, homo sapiens
GGSLSVYY

SEQ ID NO: 48 - protein, 7 aa, homo sapiens
INHSGST

SEQ ID NO: 49 - protein, 13 aa, homo sapiens
ARTSLHTWNPFDY

SEQ ID NO: 50 - protein, 6 aa, homo sapiens
QGISSY

SEQ ID NO: 51 - protein, 9 aa, homo sapiens
QQLNNYPLT

SEQ ID NO: 52 - protein, 8 aa, homo sapiens
GGTFSNYA

SEQ ID NO: 53 - protein, 8 aa, homo sapiens
IIAIFGTP

SEQ ID NO: 54 - protein, 19 aa, homo sapiens
ARRSTILERLPRHYYGMDV

SEQ ID NO: 55 - protein, 11 aa, homo sapiens
QSLLHSNGNIY

SEQ ID NO: 56 - protein, 10 aa, homo sapiens
MQTLQTLRAT

SEQ ID NO: 57 - DNA, 384 bp, homo sapiens
  CDS (1)..(384)
gaggtgcagctggtgcagtctggagtggaggtgaaaaagtccggggagtctctgaagatctcctgccggggttctggatacagttttaccagccactggatcggctgggtgcgccagatgcccgggaaaggcctggagtggatggggatcatctttcctggtgactctaagaccagatacagtccgtccttcgtaggccaggtcaccatctcagccgacaagtccatcagcaccgcctatttgcagtggagcagcctgaaggcctcggacaccgccatgtattactgtgcgagacctaatcggtattacgatgattcggggaattatgacggatcgtactactttgactactggggccagggaaccctggtcaccgtctcctca

SEQ ID NO: 58 - protein, 128 aa, homo sapiens
EVQLVQSGVEVKKSGESLKISCRGSGYSFTSHWIGWVRQMPGKGLEWMGIIFPGDSKTRYSPSFVGQVTISADKSISTAYLQWSSLKASDTAMYYCARPNRYYDDSGNYDGSYYFDYWGQGTLVTVSS

SEQ ID NO: 59 - DNA, 327 bp, homo sapiens
  CDS (1)..(327)
gaaatagtgatgacgcagtctccagccaccctgtctgtgtctccaggggaaagagccaccctctcctgcagggccagtcagagtgttaacaccaacttagcctggtaccggcagaaacctggccaggctcccaggctcctcatttatggtgcatttattaggcccactgatatcccagccaggatcactggcagtgggtctgggacagagttcactctcaccatcagcagcctgcagtcgaagattttgcagtttattactgtcaacagtataataactggcctcctgcgtggacgttcggcccagggaccaaggtggaaatcaaac

SEQ ID NO: 60 - protein, 109 aa, homo sapiens
EIVMTQSPATLSVSPGERATLSCRASQSVNTNLAWYRQKPGQAPRLLIYGAFIRPTDIPARITGSGSGTEFTLTISSLQSKILQFITVNSIITGLLRGRSAQGPRWKSN

SEQ ID NO: 61 - DNA, 357 bp, homo sapiens
  CDS (1)..(357)
caggtacagctggtgcagtctggggctgaggtgaagaagcctggggcctcagtgaaggtttcctgcaaggcatctggatacaccttcaccacctactatatgcactgggtgcgacaggcccctggacaagggcttgagtggatgggaataattaattctagtggtggcagcacaacctacgcacagaaattccggggcagagtcaccatgaccaaggacacgtccacgagcacagtgtacatggaactgagcagcctgagatctgacgacacggccgtctactactgtgcgaccagcggctggtatcgaggggcctttgactactggggccagggaaccctggtcaccgtctcctca

SEQ ID NO: 62 - protein, 119 aa, homo sapiens
QVQLVQSGAEVKKPGASVKVSCKASGYTFTTYYMHWVRQAPGQGLEWMGIINSSGGSTTYAQKFRGRVTMTKDTSTSTVYMELSSLRSDDTAVYYCATSGWYRGAFDYWGQGTLVTVSS

SEQ ID NO: 63 - DNA, 331 bp, homo sapiens
  CDS (1)..(330)
aattttatgctgactcagccgcactctgtgtcggagtctccggggaagacggtaaccatctcctgcacccgcagcagtggcagcattgacaacaactatgtacagtggtaccagcagcgcccgggcggtgcccccaccactgtgatctatgaggataaccaaagaccctctggggtccctgatcggttctctggctccttcgacagctcctccgactctgcctccctcaccatctctggactgaagactgaggacgaggctgactactactgtcagtctattgatagcaacagttgggtgttcggcggagggaccaagctgaccgtcctag

SEQ ID NO: 64 - protein, 110 aa, homo sapiens
NFMLTQPHSVSESPGKTVTISCTRSSGSIDNNYVQWYQQRPGGAPTTVIYEDNQRPSGVPDRFSGSFDSSSDSASLTISGLKTEDEADYYCQSIDSNSWVFGGGTKLTVL

SEQ ID NO: 65 - DNA, 357 bp, homo sapiens
  CDS (1)..(357)
caggttcagcttcagcagtggggcgcaggactgttgaagccttcggagaccctgtccctcacctgcgctgtctctggtgggtccttaagtgtttactactggagctggatccgccagcccccagggaaggggctggagtggattggggaaatcaatcatagtggaagcaccaactacaacccgtccctcaagagtcgagtctccatatcagtggacacgtccaagaaccagttctccctgaggctgagctctgtgaccgccgcggacacggctgtatattactgtgcgagaacttctctgcatacctggaatccctttgactactggggccagggaaccctggtcaccgtctcctca

SEQ ID NO: 66 - protein, 119 aa, homo sapiens
QVQLQQWGAGLLKPSETLSLTCAVSGGSLSVYYWSWIRQPPGKGLEWIGEINHSGSTNYNPSLKSRVSISVDTSKNQFSLRLSSVTAADTAVYYCARTSLHTWNPFDYWGQGTLVTVSS

SEQ ID NO: 67 - DNA, 322 bp, homo sapiens
  CDS (1)..(321)
gacatccagttgacccagtctccatccttcctgtctgcatctgtaggagacagagtcaccatcacttgccgggccagtcagggcattagcagttatttagcctggtatcagcaaaaaccagggaaagcccctaagctcctgatctatgctgcatccactttgcaaagtggggtcccatcaaggttcagcggcagtggatctgggacagaattcactctcacaatcagcagcctgcagcctgaagattttgcaacttattactgtcaacagcttaataattaccccctcaccttcggccaagggacacgactggagattaaac

SEQ ID NO: 68 - protein, 107 aa, homo sapiens
DIQLTQSPSFLSASVGDRVTITCRASQGISSYLAWYQQKPGKAPKLLIYAASTLQSGVPSRFSGSGSGTEFTLTISSLQPEDFATYYCQQLNNYPLTFGQGTRLEIK

SEQ ID NO: 69 - DNA, 378 bp, homo sapiens
  CDS (1)..(378)
caggtgcagctggtgcagtctggggctgaggtgaagaagcctgggtcctcggtgaaggtctcctgcaaggcttctggaggcaccttcagcaactatgctatcagctgggtgcgacaggcccctggacaagggcttgagtgggtgggagggatcatcgctatctttggtacaccaaactacgcacagaagttccagggcagagtcaccattaccgcggacgaatccacgagcacagcctacatggagctgagcagcctgagatctgaggacacggccgtgtattactgtgcgagacgttctacgattttggaacgtctgcctcgccactactacggtatggacgtctggggccaagggaccacggtcaccgtctcctca

SEQ ID NO: 70 - protein, 126 aa, homo sapiens
QVQLVQSGAEVKKPGSSVKVSCKASGGTFSNYAISWVRQAPGQGLEWVGGIIAIFGTPNYAQKFQGRVTITADESTSTAYMELSSLRSEDTAVYYCARRSTILERLPRHYYGMDVWGQGTTVTVSS

SEQ ID NO: 71 - DNA, 340 bp, homo sapiens
  CDS (1)..(339)
gaaattgtgatgactcagtctccactctccctgcccgtcacccctggagagccggcctccatctcctgcaggtctagtcagagcctcctacatagtaatggaaacatctatttggattggtatctgcagaagccagggcagtcgccacagctcctgatctatttgggttctaaccgggcctccggggtccctgacaggttcagtggcagtggatcaggcacagattttacactgaaaatcagcagagtggaggctgaggatgttggggtttattactgcatgcaaactctacaaactctccgcgcaactttcggcggagggaccaaggtggagatcaaac

SEQ ID NO: 72 - protein, 113 aa, homo sapiens
EIVMTQSPLSLPVTPGEPASISCRSSQSLLHSNGNIYLDWYLQKPGQSPQLLIYLGSNRASGVPDRFSGSGSGTDFTLKISRVEAEDVGVYYCMQTLQTLRATFGGGTKVEIK